European Patent Specification EP 3 560 515 B1, published November 15, 2023. Title: AGENT FOR IMPROVING MOTION CONTROL FUNCTION. Applicant: KAO CORPORATION. The sequence listing filed with the application follows.

SEQUENCE LISTING (5 sequences)

SEQ ID NO: 1 - DNA, 339 bp, Mus musculus
  CDS (1)..(339)
caggtccaactgcagcagcctggggctgaactggtgaagcctggggcctcagtgaagctgtcctgcaaggcttctggctacaccttcaccagcttctggatgcactgggtgattcagaggcctggacaaggccttgagtggattggagagatgaatcctagcgacggtcgtactcacttcaatgaaaagttcaagaccaaggccacactgactatagacacatcctccaacacagcctacatggaactcaacagcctgacatctgaggactctgcggtctattactgtgcaagaaggatggaggactggggccaagggactctggtcactgtttctgca

SEQ ID NO: 2 - protein, 113 aa, Mus musculus
QVQLQQPGAELVKPGASVKLSCKASGYTFTSFWMHWVIQRPGQGLEWIGEMNPSDGRTHFNEKFKTKATLTIDTSSNTAYMELNSLTSEDSAVYYCARRMEDWGQGTLVTVSA

SEQ ID NO: 3 - DNA, 324 bp, Mus musculus
  CDS (1)..(324)
gacatcaagatgacccagtctccatcttccatgtatgcatctctaggagagagagtcactatcacttgcaaggcgagtcaggacattaatagctatttaggctggttccagcagaaaccagggaaatctcctaagaccctgatatatggtgcaaacagattggtagatggggtcccatcaaggttcagtggcagtggatctgggcaagattactctctcaccatcagcagcctggagtatgacgatatgggaatatattattgtctacagtatgatgagtttccgctcaccttcggtgctgggaccaagctggagctgaaacgg

SEQ ID NO: 4 - protein, 108 aa, Mus musculus
DIKMTQSPSSMYASLGERVTITCKASQDINSYLGWFQQKPGKSPKTLIYGANRLVDGVPSRFSGSGSGQDYSLTISSLEYDDMGIYYCLQYDEFPLTFGAGTKLELKR

SEQ ID NO: 5 - protein, 42 aa, Homo sapiens
YAEGTFISDYSIAMDKIHQQDFVNWLLAQKGKKNDWKHNITQ